European Patent Specification EP 3 468 995 B1, published September 23, 2026. Title: ANTI-IGE ANTIBODIES. Applicant: UCB Biopharma sprl. The sequence listing filed with the application follows.

SEQUENCE LISTING (160 sequences)

SEQ ID NO: 1 - protein, 121 aa, Artificial Sequence [sequence omitted]

SEQ ID NO: 2 - DNA, 363 bp, Artificial Sequence
  V-region
gaagtgcagttggtggagtcgggtggagggctggtgcagcctggcggtagcctgaggctgtcctgtgccgtgtccggatactccattacctccggctactcgtggaactggatcagacaggctcccggaaagggacttgagtgggtggcgtccatcacctacgacggctcaaccaactataacccgtccgtgaagggccgcatcaccatttcgcgcgacgacagcaagaatactttttacctccaaatgaacagcctgcgggccgaagatactgccgtgtactactgcgcgcggggatcacattacttcgggcactggcacttcgccgtctggggacagggcaccctcgtcactgtctcgagc

SEQ ID NO: 3 - protein, 139 aa, Artificial Sequence
  V-region with signal sequence
MKWVTFISLLFLFSSAYSEVQLVESGGGLVQPGGSLRLSCAVSGYSITSGYSWNWIRQAPGKGLEWVASITYDGSTNYNPSVKGRITISRDDSKNTFYLQMNSLRAEDTAVYYCARGSHYFGHWHFAVWGQGTLVTVSS

SEQ ID NO: 4 - DNA, 417 bp, Artificial Sequence
  V-region with signal sequence
atgaagtgggtcaccttcatctccctgctgtttctgttctccagcgcctactccgaagtgcagttggtggagtcgggtggagggctggtgcagcctggcggtagcctgaggctgtcctgtgccgtgtccggatactccattacctccggctactcgtggaactggatcagacaggctcccggaaagggacttgagtgggtggcgtccatcacctacgacggctcaaccaactataacccgtccgtgaagggccgcatcaccatttcgcgcgacgacagcaagaatactttttacctccaaatgaacagcctgcgggccgaagatactgccgtgtactactgcgcgcggggatcacattacttcgggcactggcacttcgccgtctggggacagggcaccctcgtcactgtctcgagc

SEQ ID NO: 5 - protein, 224 aa, Artificial Sequence
  v-region + gamma 1 CH1 constant region
EVQLVESGGGLVQPGGSLRLSCAVSGYSITSGYSWNWIRQAPGKGLEWVASITYDGSTNYNPSVKGRITISRDDSKNTFYLQMNSLRAEDTAVYYCARGSHYFGHWHFAVWGQGTLVTVSSASTKGPSVFPLAPSSKSTSGGTAALGCLVKDYFPEPVTVSWNSGALTSGVHTFPAVLQSSGLYSLSSVVTVPSSSLGTQTYICNVNHKPSNTKVDKKVEPKSC

SEQ ID NO: 6 - DNA, 672 bp, Artificial Sequence
  v-region + gamma 1 CH1 constant region
gaagtgcagttggtggagtcgggtggagggctggtgcagcctggcggtagcctgaggctgtcctgtgccgtgtccggatactccattacctccggctactcgtggaactggatcagacaggctcccggaaagggacttgagtgggtggcgtccatcacctacgacggctcaaccaactataacccgtccgtgaagggccgcatcaccatttcgcgcgacgacagcaagaatactttttacctccaaatgaacagcctgcgggccgaagatactgccgtgtactactgcgcgcggggatcacattacttcgggcactggcacttcgccgtctggggacagggcaccctcgtcactgtctcgagcgcttctacaaagggcccatcggtcttccccctggcaccctcctccaagagcacctctgggggcacagcggccctgggctgcctggtcaaggactacttccccgaaccggtgacggtgtcgtggaactcaggcgccctgaccagcggcgtgcacaccttcccggctgtcctacagtcctcaggactctactccctcagcagcgtggtgaccgtgccctccagcagcttgggcacccagacctacatctgcaacgtgaatcacaagcccagcaacaccaaggtggacaagaaagttgagcccaaatcttgt

SEQ ID NO: 7 - protein, 242 aa, Artificial Sequence
  v-region + gamma 1 CH1 constant region with signal sequence
MKWVTFISLLFLFSSAYSEVQLVESGGGLVQPGGSLRLSCAVSGYSITSGYSWNWIRQAPGKGLEWVASITYDGSTNYNPSVKGRITISRDDSKNTFYLQMNSLRAEDTAVYYCARGSHYFGHWHFAVWGQGTLVTVSSASTKGPSVFPLAPSSKSTSGGTAALGCLVKDYFPEPVTVSWNSGALTSGVHTFPAVLQSSGLYSLSSVVTVPSSSLGTQTYICNVNHKPSNTKVDKKVEPKSC

SEQ ID NO: 8 - DNA, 726 bp, Artificial Sequence
  v-region + gamma 1 CH1 constant region with signal sequence
atgaagtgggtcaccttcatctccctgctgtttctgttctccagcgcctactccgaagtgcagttggtggagtcgggtggagggctggtgcagcctggcggtagcctgaggctgtcctgtgccgtgtccggatactccattacctccggctactcgtggaactggatcagacaggctcccggaaagggacttgagtgggtggcgtccatcacctacgacggctcaaccaactataacccgtccgtgaagggccgcatcaccatttcgcgcgacgacagcaagaatactttttacctccaaatgaacagcctgcgggccgaagatactgccgtgtactactgcgcgcggggatcacattacttcgggcactggcacttcgccgtctggggacagggcaccctcgtcactgtctcgagcgcttctacaaagggcccatcggtcttccccctggcaccctcctccaagagcacctctgggggcacagcggccctgggctgcctggtcaaggactacttccccgaaccggtgacggtgtcgtggaactcaggcgccctgaccagcggcgtgcacaccttcccggctgtcctacagtcctcaggactctactccctcagcagcgtggtgaccgtgccctccagcagcttgggcacccagacctacatctgcaacgtgaatcacaagcccagcaacaccaaggtggacaagaaagttgagcccaaatcttgt

SEQ ID NO: 9 - protein, 451 aa, Artificial Sequence
  v-region + gamma 1 full length constant region
EVQLVESGGGLVQPGGSLRLSCAVSGYSITSGYSWNWIRQAPGKGLEWVASITYDGSTNYNPSVKGRITISRDDSKNTFYLQMNSLRAEDTAVYYCARGSHYFGHWHFAVWGQGTLVTVSSASTKGPSVFPLAPSSKSTSGGTAALGCLVKDYFPEPVTVSWNSGALTSGVHTFPAVLQSSGLYSLSSVVTVPSSSLGTQTYICNVNHKPSNTKVDKKVEPKSCDKTHTCPPCPAPELLGGPSVFLFPPKPKDTLMISRTPEVTCVVVDVSHEDPEVKFNWYVDGVEVHNAKTKPREEQYNSTYRVVSVLTVLHQDWLNGKEYKCKVSNKALPAPIEKTISKAKGQPREPQVYTLPPSREEMTKNQVSLTCLVKGFYPSDIAVEWESNGQPENNYKTTPPVLDSDGSFFLYSKLTVDKSRWQQGNVFSCSVMHEALHNHYTQKSLSLSPGK

SEQ ID NO: 10 - DNA, 1353 bp, Artificial Sequence
  v-region + gamma 1 full length constant region
gaagtgcagttggtggagtcgggtggagggctggtgcagcctggcggtagcctgaggctgtcctgtgccgtgtccggatactccattacctccggctactcgtggaactggatcagacaggctcccggaaagggacttgagtgggtggcgtccatcacctacgacggctcaaccaactataacccgtccgtgaagggccgcatcaccatttcgcgcgacgacagcaagaatactttttacctccaaatgaacagcctgcgggccgaagatactgccgtgtactactgcgcgcggggatcacattacttcgggcactggcacttcgccgtctggggacagggcaccctcgtcactgtctcgagcgcttctacaaagggcccctccgtgttcccgctcgctccatcatcgaagtctaccagcggaggcactgcggctctcggttgcctcgtgaaggactacttcccggagccggtgaccgtgtcgtggaacagcggagccctgaccagcggggtgcacacctttccggccgtcttgcagtcaagcggcctttactccctgtcatcagtggtgactgtcccgtccagctcattgggaacccaaacctacatctgcaatgtgaatcacaaacctagcaacaccaaggttgacaagaaagtcgagcccaaatcgtgtgacaagactcacacttgtccgccgtgcccggcacccgaactgctgggaggtcccagcgtctttctgttccctccaaagccgaaagacacgctgatgatctcccgcaccccggaggtcacttgcgtggtcgtggacgtgtcacatgaggacccagaggtgaagttcaattggtacgtggatggcgtcgaagtccacaatgccaaaactaagcccagagaagaacagtacaattcgacctaccgcgtcgtgtccgtgctcacggtgttgcatcaggattggctgaacgggaaggaatacaagtgcaaagtgtccaacaaggcgctgccggcaccgatcgagaaaactatctccaaagcgaagggacagcctagggaacctcaagtctacacgctgccaccatcacgggaagaaatgactaagaatcaagtctcactgacttgtctggtgaaggggttttaccctagcgacattgccgtggagtgggaatccaacggccagccagagaacaactacaagactacccctccagtgctcgactcggatggatcgttcttcctttactcgaagctcaccgtggataagtcccggtggcagcagggaaacgtgttctcctgctcggtgatgcatgaagccctccataaccactatacccaaaagtcgctgtccctgtcgccgggaaag

SEQ ID NO: 11 - protein, 469 aa, Artificial Sequence
  v-region + gamma 1 full length constant region with signal sequence
MKWVTFISLLFLFSSAYSEVQLVESGGGLVQPGGSLRLSCAVSGYSITSGYSWNWIRQAPGKGLEWVASITYDGSTNYNPSVKGRITISRDDSKNTFYLQMNSLRAEDTAVYYCARGSHYFGHWHFAVWGQGTLVTVSSASTKGPSVFPLAPSSKSTSGGTAALGCLVKDYFPEPVTVSWNSGALTSGVHTFPAVLQSSGLYSLSSVVTVPSSSLGTQTYICNVNHKPSNTKVDKKVEPKSCDKTHTCPPCPAPELLGGPSVFLFPPKPKDTLMISRTPEVTCVVVDVSHEDPEVKFNWYVDGVEVHNAKTKPREEQYNSTYRVVSVLTVLHQDWLNGKEYKCKVSNKALPAPIEKTISKAKGQPREPQVYTLPPSREEMTKNQVSLTCLVKGFYPSDIAVEWESNGQPENNYKTTPPVLDSDGSFFLYSKLTVDKSRWQQGNVFSCSVMHEALHNHYTQKSLSLSPGK

SEQ ID NO: 12 - DNA, 1407 bp, Artificial Sequence
  v-region + gamma 1 full length constant region with signal sequence
atgaagtgggtcaccttcatctccctgctgtttctgttctccagcgcctactccgaagtgcagttggtggagtcgggtggagggctggtgcagcctggcggtagcctgaggctgtcctgtgccgtgtccggatactccattacctccggctactcgtggaactggatcagacaggctcccggaaagggacttgagtgggtggcgtccatcacctacgacggctcaaccaactataacccgtccgtgaagggccgcatcaccatttcgcgcgacgacagcaagaatactttttacctccaaatgaacagcctgcgggccgaagatactgccgtgtactactgcgcgcggggatcacattacttcgggcactggcacttcgccgtctggggacagggcaccctcgtcactgtctcgagcgcttctacaaagggcccctccgtgttcccgctcgctccatcatcgaagtctaccagcggaggcactgcggctctcggttgcctcgtgaaggactacttcccggagccggtgaccgtgtcgtggaacagcggagccctgaccagcggggtgcacacctttccggccgtcttgcagtcaagcggcctttactccctgtcatcagtggtgactgtcccgtccagctcattgggaacccaaacctacatctgcaatgtgaatcacaaacctagcaacaccaaggttgacaagaaagtcgagcccaaatcgtgtgacaagactcacacttgtccgccgtgcccggcacccgaactgctgggaggtcccagcgtctttctgttccctccaaagccgaaagacacgctgatgatctcccgcaccccggaggtcacttgcgtggtcgtggacgtgtcacatgaggacccagaggtgaagttcaattggtacgtggatggcgtcgaagtccacaatgccaaaactaagcccagagaagaacagtacaattcgacctaccgcgtcgtgtccgtgctcacggtgttgcatcaggattggctgaacgggaaggaatacaagtgcaaagtgtccaacaaggcgctgccggcaccgatcgagaaaactatctccaaagcgaagggacagcctagggaacctcaagtctacacgctgccaccatcacgggaagaaatgactaagaatcaagtctcactgacttgtctggtgaaggggttttaccctagcgacattgccgtggagtgggaatccaacggccagccagagaacaactacaagactacccctccagtgctcgactcggatggatcgttcttcctttactcgaagctcaccgtggataagtcccggtggcagcagggaaacgtgttctcctgctcggtgatgcatgaagccctccataaccactatacccaaaagtcgctgtccctgtcgccgggaaag

SEQ ID NO: 13 - protein, 25 aa, Artificial Sequence [sequence omitted]

SEQ ID NO: 14 - protein, 11 aa, Artificial Sequence
  CDRH1
GYSITSGYSWN

SEQ ID NO: 15 - protein, 14 aa, Artificial Sequence
  FR H2
WIRQAPGKGLEWVA

SEQ ID NO: 16 - protein, 16 aa, Artificial Sequence
  CDRH2
SITYDGSTNYNPSVKG

SEQ ID NO: 17 - protein, 32 aa, Artificial Sequence
  FR H3
RITISRDDSKNTFYLQMNSLRAEDTAVYYCAR

SEQ ID NO: 18 - protein, 12 aa, Artificial Sequence
  CDRH3
GSHYFGHWHFAV

SEQ ID NO: 19 - protein, 11 aa, Artificial Sequence
  FR H4
WGQGTLVTVSS

SEQ ID NO: 20 - protein, 111 aa, Artificial Sequence [sequence omitted]

SEQ ID NO: 21 - DNA, 333 bp, Artificial Sequence
  V-region light
gatattcagctgactcagagcccgagctcactctccgcttccgtgggggatagagtgaccatcacttgccgggcatcccagtcggtggactacgacggagactcctacatgaactggtatcagcagaagcccggaaaagccccaaagttgctgatctacgccgcctcataccttgaaagcggcgtgccttcgcgcttctcgggaagcgggtcgggcaccgatttcaccctgaccatttcgtcgctgcagccggaggacttcgcgacttactactgccaacagtcccacgaggacccctatacgtttggccagggaaccaaggtcgaaatcaag

SEQ ID NO: 22 - protein, 129 aa, Artificial Sequence
  V-region light with signal sequence
MKWVTFISLLFLFSSAYSDIQLTQSPSSLSASVGDRVTITCRASQSVDYDGDSYMNWYQQKPGKAPKLLIYAASYLESGVPSRFSGSGSGTDFTLTISSLQPEDFATYYCQQSHEDPYTFGQGTKVEIK

SEQ ID NO: 23 - DNA, 387 bp, Artificial Sequence
  V-region light with signal sequence
atgaagtgggtcaccttcatctccctgctgtttctgttctcctccgcctactccgatattcagctgactcagagcccgagctcactctccgcttccgtgggggatagagtgaccatcacttgccgggcatcccagtcggtggactacgacggagactcctacatgaactggtatcagcagaagcccggaaaagccccaaagttgctgatctacgccgcctcataccttgaaagcggcgtgccttcgcgcttctcgggaagcgggtcgggcaccgatttcaccctgaccatttcgtcgctgcagccggaggacttcgcgacttactactgccaacagtcccacgaggacccctatacgtttggccagggaaccaaggtcgaaatcaag

SEQ ID NO: 24 - protein, 218 aa, Artificial Sequence
  V-region light + kappa constant region
DIQLTQSPSSLSASVGDRVTITCRASQSVDYDGDSYMNWYQQKPGKAPKLLIYAASYLESGVPSRFSGSGSGTDFTLTISSLQPEDFATYYCQQSHEDPYTFGQGTKVEIKRTVAAPSVFIFPPSDEQLKSGTASVVCLLNNFYPREAKVQWKVDNALQSGNSQESVTEQDSKDSTYSLSSTLTLSKADYEKHKVYACEVTHQGLSSPVTKSFNRGEC

SEQ ID NO: 25 - DNA, 654 bp, Artificial Sequence
  V-region + kappa constant region
gatattcagctgactcagagcccgagctcactctccgcttccgtgggggatagagtgaccatcacttgccgggcatcccagtcggtggactacgacggagactcctacatgaactggtatcagcagaagcccggaaaagccccaaagttgctgatctacgccgcctcataccttgaaagcggcgtgccttcgcgcttctcgggaagcgggtcgggcaccgatttcaccctgaccatttcgtcgctgcagccggaggacttcgcgacttactactgccaacagtcccacgaggacccctatacgtttggccagggaaccaaggtcgaaatcaagcgtacggtagcggccccatctgtcttcatcttcccgccatctgatgagcagttgaaatctggaactgcctctgttgtgtgcctgctgaataacttctatcccagagaggccaaagtacagtggaaggtggataacgccctccaatcgggtaactcccaggagagtgtcacagagcaggacagcaaggacagcacctacagcctcagcagcaccctgacgctgagcaaagcagactacgagaaacacaaagtctacgcctgcgaagtcacccatcagggcctgagctcgcccgtcacaaagagcttcaacaggggagagtgt

SEQ ID NO: 26 - protein, 236 aa, Artificial Sequence
  V-region + kappa constant region with signal sequence
MKWVTFISLLFLFSSAYSDIQLTQSPSSLSASVGDRVTITCRASQSVDYDGDSYMNWYQQKPGKAPKLLIYAASYLESGVPSRFSGSGSGTDFTLTISSLQPEDFATYYCQQSHEDPYTFGQGTKVEIKRTVAAPSVFIFPPSDEQLKSGTASVVCLLNNFYPREAKVQWKVDNALQSGNSQESVTEQDSKDSTYSLSSTLTLSKADYEKHKVYACEVTHQGLSSPVTKSFNRGEC

SEQ ID NO: 27 - DNA, 708 bp, Artificial Sequence
  V-region + kappa constant region with signal seque
atgaagtgggtcaccttcatctccctgctgtttctgttctcctccgcctactccgatattcagctgactcagagcccgagctcactctccgcttccgtgggggatagagtgaccatcacttgccgggcatcccagtcggtggactacgacggagactcctacatgaactggtatcagcagaagcccggaaaagccccaaagttgctgatctacgccgcctcataccttgaaagcggcgtgccttcgcgcttctcgggaagcgggtcgggcaccgatttcaccctgaccatttcgtcgctgcagccggaggacttcgcgacttactactgccaacagtcccacgaggacccctatacgtttggccagggaaccaaggtcgaaatcaagcgtacggtagcggccccatctgtcttcatcttcccgccatctgatgagcagttgaaatctggaactgcctctgttgtgtgcctgctgaataacttctatcccagagaggccaaagtacagtggaaggtggataacgccctccaatcgggtaactcccaggagagtgtcacagagcaggacagcaaggacagcacctacagcctcagcagcaccctgacgctgagcaaagcagactacgagaaacacaaagtctacgcctgcgaagtcacccatcagggcctgagctcgcccgtcacaaagagcttcaacaggggagagtgt

SEQ ID NO: 28 - protein, 23 aa, Artificial Sequence
  FR L1
DIQLTQSPSSLSASVGDRVTITC

SEQ ID NO: 29 - protein, 15 aa, Artificial Sequence
  CDRL1
RASQSVDYDGDSYMN

SEQ ID NO: 30 - protein, 15 aa, Artificial Sequence
  FR L2
WYQQKPGKAPKLLIY

SEQ ID NO: 31 - protein, 7 aa, Artificial Sequence
  CDRL2
AASYLES

SEQ ID NO: 32 - protein, 32 aa, Artificial Sequence
  FR L3
GVPSRFSGSGSGTDFTLTISSLQPEDFATYYC

SEQ ID NO: 33 - protein, 9 aa, Artificial Sequence
  CDRL3
QQSHEDPYT

SEQ ID NO: 34 - protein, 10 aa, Artificial Sequence
  FR L4
FGQGTKVEIK

SEQ ID NO: 35 - protein, 111 aa, Artificial Sequence
  S60M_S77R_Q79R_v-region
DIQLTQSPSSLSASVGDRVTITCRASQSVDYDGDSYMNWYQQKPGKAPKLLIYAASYLESGVPMRFSGSGSGTDFTLTISRLRPEDFATYYCQQSHEDPYTFGQGTKVEIK

SEQ ID NO: 36 - DNA, 333 bp, Artificial Sequence
  S60M_S77R_Q79R_v-region
gatattcagctgactcagagcccgagctcactctccgcttccgtgggggatagagtgaccatcacttgccgggcatcccagtcggtggactacgacggagactcctacatgaactggtatcagcagaagcccggaaaagccccaaagttgctgatctacgccgcctcataccttgaaagcggcgtgcctatgcgcttctcgggaagcgggtcgggcaccgatttcaccctgaccatttcgagactgaggccggaggacttcgcgacttactactgccaacagtcccacgaggacccctatacgtttggccagggaaccaaggtcgaaatcaag

SEQ ID NO: 37 - protein, 129 aa, Artificial Sequence
  S60M_S77R_Q79R_v-region with signal sequence
MKWVTFISLLFLFSSAYSDIQLTQSPSSLSASVGDRVTITCRASQSVDYDGDSYMNWYQQKPGKAPKLLIYAASYLESGVPMRFSGSGSGTDFTLTISRLRPEDFATYYCQQSHEDPYTFGQGTKVEIK

SEQ ID NO: 38 - DNA, 387 bp, Artificial Sequence
  S60M_S77R_Q79R_v-region with signal sequence
atgaagtgggtcaccttcatctccctgctgtttctgttctcctccgcctactccgatattcagctgactcagagcccgagctcactctccgcttccgtgggggatagagtgaccatcacttgccgggcatcccagtcggtggactacgacggagactcctacatgaactggtatcagcagaagcccggaaaagccccaaagttgctgatctacgccgcctcataccttgaaagcggcgtgcctatgcgcttctcgggaagcgggtcgggcaccgatttcaccctgaccatttcgagactgaggccggaggacttcgcgacttactactgccaacagtcccacgaggacccctatacgtttggccagggaaccaaggtcgaaatcaag

SEQ ID NO: 39 - protein, 218 aa, Artificial Sequence
  S60M_S77R_Q79R_v-region + kappa constant region including L154P
DIQLTQSPSSLSASVGDRVTITCRASQSVDYDGDSYMNWYQQKPGKAPKLLIYAASYLESGVPMRFSGSGSGTDFTLTISRLRPEDFATYYCQQSHEDPYTFGQGTKVEIKRTVAAPSVFIFPPSDEQLKSGTASVVCLLNNFYPREAKVQWKVDNAPQSGNSQESVTEQDSKDSTYSLSSTLTLSKADYEKHKVYACEVTHQGLSSPVTKSFNRGEC

SEQ ID NO: 40 - DNA, 654 bp, Artificial Sequence
  S60M_S77R_Q79R_v-region + kappa constant region including L154P
gatattcagctgactcagagcccgagctcactctccgcttccgtgggggatagagtgaccatcacttgccgggcatcccagtcggtggactacgacggagactcctacatgaactggtatcagcagaagcccggaaaagccccaaagttgctgatctacgccgcctcataccttgaaagcggcgtgcctatgcgcttctcgggaagcgggtcgggcaccgatttcaccctgaccatttcgagactgaggccggaggacttcgcgacttactactgccaacagtcccacgaggacccctatacgtttggccagggaaccaaggtcgaaatcaagcgtacggtagcggccccatctgtcttcatcttcccgccatctgatgagcagttgaaatctggaactgcctctgttgtgtgcctgctgaataacttctatcccagagaggccaaagtacagtggaaggtggataacgccccgcaatcgggtaactcccaggagagtgtcacagagcaggacagcaaggacagcacctacagcctcagcagcaccctgacgctgagcaaagcagactacgagaaacacaaagtctacgcctgcgaagtcacccatcagggcctgagctcgcccgtcacaaagagcttcaacaggggagagtgt

SEQ ID NO: 41 - protein, 236 aa, Artificial Sequence
  S60M_S77R_Q79R_v-region + kappa constant region including L154P with signal sequence
MKWVTFISLLFLFSSAYSDIQLTQSPSSLSASVGDRVTITCRASQSVDYDGDSYMNWYQQKPGKAPKLLIYAASYLESGVPMRFSGSGSGTDFTLTISRLRPEDFATYYCQQSHEDPYTFGQGTKVEIKRTVAAPSVFIFPPSDEQLKSGTASVVCLLNNFYPREAKVQWKVDNAPQSGNSQESVTEQDSKDSTYSLSSTLTLSKADYEKHKVYACEVTHQGLSSPVTKSFNRGEC

SEQ ID NO: 42 - DNA, 708 bp, Artificial Sequence
  S60M_S77R_Q79R_v-region + kappa constant region including L154P with signal sequence
atgaagtgggtcaccttcatctccctgctgtttctgttctcctccgcctactccgatattcagctgactcagagcccgagctcactctccgcttccgtgggggatagagtgaccatcacttgccgggcatcccagtcggtggactacgacggagactcctacatgaactggtatcagcagaagcccggaaaagccccaaagttgctgatctacgccgcctcataccttgaaagcggcgtgcctatgcgcttctcgggaagcgggtcgggcaccgatttcaccctgaccatttcgagactgaggccggaggacttcgcgacttactactgccaacagtcccacgaggacccctatacgtttggccagggaaccaaggtcgaaatcaagcgtacggtagcggccccatctgtcttcatcttcccgccatctgatgagcagttgaaatctggaactgcctctgttgtgtgcctgctgaataacttctatcccagagaggccaaagtacagtggaaggtggataacgccccgcaatcgggtaactcccaggagagtgtcacagagcaggacagcaaggacagcacctacagcctcagcagcaccctgacgctgagcaaagcagactacgagaaacacaaagtctacgcctgcgaagtcacccatcagggcctgagctcgcccgtcacaaagagcttcaacaggggagagtgt

SEQ ID NO: 43 - protein, 32 aa, Artificial Sequence
  FR L3 S64M  S60M
GVPMRFSGSGSGTDFTLTISSLQPEDFATYYC

SEQ ID NO: 44 - protein, 32 aa, Artificial Sequence
  FR L3 S81R S77R
GVPSRFSGSGSGTDFTLTISRLQPEDFATYYC

SEQ ID NO: 45 - protein, 32 aa, Artificial Sequence
  FR L3 Q83R Q79R
GVPSRFSGSGSGTDFTLTISSLRPEDFATYYC

SEQ ID NO: 46 - protein, 32 aa, Artificial Sequence
  FR L3 S64M S81R S60M S77R
GVPMRFSGSGSGTDFTLTISRLQPEDFATYYC

SEQ ID NO: 47 - protein, 32 aa, Artificial Sequence
  FR L3 S64M Q83R S60M Q79R
GVPMRFSGSGSGTDFTLTISSLRPEDFATYYC

SEQ ID NO: 48 - protein, 32 aa, Artificial Sequence
  FR L3 S81R Q83R S77R Q79R
GVPSRFSGSGSGTDFTLTISRLRPEDFATYYC

SEQ ID NO: 49 - protein, 32 aa, Artificial Sequence
  FR L3 S64M S81R Q83R S60M S77R Q79R
GVPMRFSGSGSGTDFTLTISRLRPEDFATYYC

SEQ ID NO: 50 - protein, 7 aa, Artificial Sequence
  CDRL2 S56D S52D
AADYLES

SEQ ID NO: 51 - protein, 7 aa, Artificial Sequence
  CDRL2 S56E S52E
AAEYLES

SEQ ID NO: 52 - protein, 32 aa, Artificial Sequence
  FR L3 S71M S67M
GVPSRFSGSGMGTDFTLTISSLQPEDFATYYC

SEQ ID NO: 53 - protein, 32 aa, Artificial Sequence
  FR L3 S64M S71M S60M S67M
GVPMRFSGSGMGTDFTLTISSLQPEDFATYYC

SEQ ID NO: 54 - protein, 32 aa, Artificial Sequence
  FR L3 S81R S71M S77R S67M
GVPSRFSGSGMGTDFTLTISRLQPEDFATYYC

SEQ ID NO: 55 - protein, 32 aa, Artificial Sequence
  FR L3 Q83R S71M Q79R S67M
GVPSRFSGSGMGTDFTLTISSLRPEDFATYYC

SEQ ID NO: 56 - protein, 32 aa, Artificial Sequence
  FR L3 S64M S81R S71M S60M S77R S67M
GVPMRFSGSGMGTDFTLTISRLQPEDFATYYC

SEQ ID NO: 57 - protein, 32 aa, Artificial Sequence
  FR L3 S64M Q83R S71M S60M Q79R S67M
GVPMRFSGSGMGTDFTLTISSLRPEDFATYYC

SEQ ID NO: 58 - protein, 32 aa, Artificial Sequence
  FR L3 S81R Q83R S71M S77R Q79R S67M
GVPSRFSGSGMGTDFTLTISRLRPEDFATYYC

SEQ ID NO: 59 - protein, 32 aa, Artificial Sequence
  FR L3 S64M S81R Q83R S71M S60M S77R Q79R S67M
GVPMRFSGSGMGTDFTLTISRLRPEDFATYYC

SEQ ID NO: 60 - protein, 32 aa, Artificial Sequence
  FR L3 S67Y S63Y
GVPSRFYGSGSGTDFTLTISSLQPEDFATYYC

SEQ ID NO: 61 - protein, 32 aa, Artificial Sequence
  FR L3 S64M S67Y S60M S63Y
GVPMRFYGSGSGTDFTLTISSLQPEDFATYYC

SEQ ID NO: 62 - protein, 32 aa, Artificial Sequence
  FR L3 S81R S67Y S77R S63Y
GVPSRFYGSGSGTDFTLTISRLQPEDFATYYC

SEQ ID NO: 63 - protein, 32 aa, Artificial Sequence
  FR L3 Q83R S67Y Q79R S63Y
GVPSRFYGSGSGTDFTLTISSLRPEDFATYYC

SEQ ID NO: 64 - protein, 32 aa, Artificial Sequence
  FR L3 S64M S81R S67Y S60M S77R S63Y
GVPMRFYGSGSGTDFTLTISRLQPEDFATYYC

SEQ ID NO: 65 - protein, 32 aa, Artificial Sequence
  FR L3 S64M Q83R S67Y S60M Q79R S63Y
GVPMRFYGSGSGTDFTLTISSLRPEDFATYYC

SEQ ID NO: 66 - protein, 32 aa, Artificial Sequence
  FR L3 S81R Q83R S67Y S77R Q79R S63Y
GVPSRFYGSGSGTDFTLTISRLRPEDFATYYC

SEQ ID NO: 67 - protein, 32 aa, Artificial Sequence
  FR L3 S64M S81R Q83R S67Y S60M S77R Q79R S63Y
GVPMRFYGSGSGTDFTLTISRLRPEDFATYYC

SEQ ID NO: 68 - protein, 32 aa, Artificial Sequence
  FR L3 S80N S76N
GVPSRFSGSGSGTDFTLTINSLQPEDFATYYC

SEQ ID NO: 69 - protein, 32 aa, Artificial Sequence
  FR L3 S64M S80N S60M S76N
GVPMRFSGSGSGTDFTLTINSLQPEDFATYYC

SEQ ID NO: 70 - protein, 32 aa, Artificial Sequence
  FR L3 S81R S80N S77R S76
GVPSRFSGSGSGTDFTLTINRLQPEDFATYYC

SEQ ID NO: 71 - protein, 32 aa, Artificial Sequence
  FR L3 Q83R S80N Q79R S76N
GVPSRFSGSGSGTDFTLTINSLRPEDFATYYC

SEQ ID NO: 72 - protein, 32 aa, Artificial Sequence
  FR L3 S64M S81R S80N S60M S77R S76N
GVPMRFSGSGSGTDFTLTINRLQPEDFATYYC

SEQ ID NO: 73 - protein, 32 aa, Artificial Sequence
  FR L3 S64M Q83R S80N S60M Q79R S76N
GVPMRFSGSGSGTDFTLTINSLRPEDFATYYC

SEQ ID NO: 74 - protein, 32 aa, Artificial Sequence
  FR L3 S81R Q83R S80N S77R Q79R S76N
GVPSRFSGSGSGTDFTLTINRLRPEDFATYYC

SEQ ID NO: 75 - protein, 32 aa, Artificial Sequence
  FR L3 S64M S81R Q83R S80N S60M S77R Q79R S76N
GVPMRFSGSGSGTDFTLTINRLRPEDFATYYC

SEQ ID NO: 76 - protein, 32 aa, Artificial Sequence
  FR L3 S80N S67Y S76N S63Y
GVPSRFYGSGSGTDFTLTINSLQPEDFATYYC

SEQ ID NO: 77 - protein, 32 aa, Artificial Sequence
  FR L3 S64M S80N S67Y S60M S76N S63Y
GVPMRFYGSGSGTDFTLTINSLQPEDFATYYC

SEQ ID NO: 78 - protein, 32 aa, Artificial Sequence
  FR L3 S81R S80N S67Y S77R S76N S63Y
GVPSRFYGSGSGTDFTLTINRLQPEDFATYYC

SEQ ID NO: 79 - protein, 32 aa, Artificial Sequence
  FR L3 Q83R S80N S67Y Q79R S76N S63Y
GVPSRFYGSGSGTDFTLTINSLRPEDFATYYC

SEQ ID NO: 80 - protein, 32 aa, Artificial Sequence
  FR L3 S64M S81R S80N S67Y S60M S77R S76N S63Y
GVPMRFYGSGSGTDFTLTINRLQPEDFATYYC

SEQ ID NO: 81 - protein, 32 aa, Artificial Sequence
  FR L3 S64M Q83R S80N S67Y S60M Q79R S76N S63Y
GVPMRFYGSGSGTDFTLTINSLRPEDFATYYC

SEQ ID NO: 82 - protein, 32 aa, Artificial Sequence
  FR L3 S81R Q83R S80N S67Y S77R Q79R S76N S63Y
GVPSRFYGSGSGTDFTLTINRLRPEDFATYYC

SEQ ID NO: 83 - protein, 32 aa, Artificial Sequence
  FR L3 S64M S81R Q83R S80N S67Y S60M S77R Q79R S76N S63Y
GVPMRFYGSGSGTDFTLTINRLRPEDFATYYC

SEQ ID NO: 84 - protein, 32 aa, Artificial Sequence
  FR L3 S67Y S71M S63Y S67M
GVPSRFYGSGMGTDFTLTISSLQPEDFATYYC

SEQ ID NO: 85 - protein, 32 aa, Artificial Sequence
  FR L3 S64M S67Y S71M S60M S63Y S67M
GVPMRFYGSGMGTDFTLTISSLQPEDFATYYC

SEQ ID NO: 86 - protein, 32 aa, Artificial Sequence
  FR L3 S81R S67Y S71M S77R S63Y S67M
GVPSRFYGSGMGTDFTLTISRLQPEDFATYYC

SEQ ID NO: 87 - protein, 32 aa, Artificial Sequence
  FR L3 Q83R S67Y S71M Q79R S63Y S67M
GVPSRFYGSGMGTDFTLTISSLRPEDFATYYC

SEQ ID NO: 88 - protein, 32 aa, Artificial Sequence
  FR L3 S64M S81R S67Y S71M S60M S77R S63Y S67M
GVPMRFYGSGMGTDFTLTISRLQPEDFATYYC

SEQ ID NO: 89 - protein, 32 aa, Artificial Sequence
  FR L3 S64M Q83R S67Y S71M S60M Q79R S63Y S67M
GVPMRFYGSGMGTDFTLTISSLRPEDFATYYC

SEQ ID NO: 90 - protein, 32 aa, Artificial Sequence
  FR L3 S81R Q83R S67Y S71M S77R Q79R S63Y S67M
GVPSRFYGSGMGTDFTLTISRLRPEDFATYYC

SEQ ID NO: 91 - protein, 32 aa, Artificial Sequence
  FR L3 S64M S81R Q83R S67Y S71M S60M S77R Q79R S63Y S67M
GVPMRFYGSGMGTDFTLTISRLRPEDFATYYC

SEQ ID NO: 92 - protein, 32 aa, Artificial Sequence
  FR L3 S80N S71M S76N S67M
GVPSRFSGSGMGTDFTLTINSLQPEDFATYYC

SEQ ID NO: 93 - protein, 32 aa, Artificial Sequence
  FR L3 S64M S80N S71M S60M S76N S67M (
GVPMRFSGSGMGTDFTLTINSLQPEDFATYYC

SEQ ID NO: 94 - protein, 32 aa, Artificial Sequence
  FR L3 S81R S80N S71M S77R S76N S67M
GVPSRFSGSGMGTDFTLTINRLQPEDFATYYC

SEQ ID NO: 95 - protein, 32 aa, Artificial Sequence
  FR L3 Q83R S80N S71M Q79R S76N S67M
GVPSRFSGSGMGTDFTLTINSLRPEDFATYYC

SEQ ID NO: 96 - protein, 32 aa, Artificial Sequence
  FR L3 S64M S81R S80N S71M S60M S77R S76N S67M
GVPMRFSGSGMGTDFTLTINRLQPEDFATYYC

SEQ ID NO: 97 - protein, 32 aa, Artificial Sequence
  FR L3 S64M Q83R S80N S71M S60M Q79R S76N S67M
GVPMRFSGSGMGTDFTLTINSLRPEDFATYYC

SEQ ID NO: 98 - protein, 32 aa, Artificial Sequence
  FR L3 S81R Q83R S80N S71M S77R Q79R S76N S67M
GVPSRFSGSGMGTDFTLTINRLRPEDFATYYC

SEQ ID NO: 99 - protein, 32 aa, Artificial Sequence
  FR L3 S64M S81R Q83R S80N S71M S60M S77R Q79R S76N S67M
GVPMRFSGSGMGTDFTLTINRLRPEDFATYYC

SEQ ID NO: 100 - protein, 32 aa, Artificial Sequence
  FR L3 S80N S67Y S71M S76N S63Y S67M
GVPSRFYGSGMGTDFTLTINSLQPEDFATYYC

SEQ ID NO: 101 - protein, 32 aa, Artificial Sequence
  FR L3 S64M S80N S67Y S71M S60M S76N S63Y S67M
GVPMRFYGSGMGTDFTLTINSLQPEDFATYYC

SEQ ID NO: 102 - protein, 32 aa, Artificial Sequence
  FR L3 S81R S80N S67Y S71M S77R S76N S63Y S67M
GVPSRFYGSGMGTDFTLTINRLQPEDFATYYC

SEQ ID NO: 103 - protein, 32 aa, Artificial Sequence
  FR L3 Q83R S80N S67Y S71M Q79R S76N S63Y S67M
GVPSRFYGSGMGTDFTLTINSLRPEDFATYYC

SEQ ID NO: 104 - protein, 32 aa, Artificial Sequence
  FR L3 S64M S81R S80N S67Y S71M S60M S77R S76N S63Y S67M
GVPMRFYGSGMGTDFTLTINRLQPEDFATYYC

SEQ ID NO: 105 - protein, 32 aa, Artificial Sequence
  FR L3 S64M Q83R S80N S67Y S71M S60M Q79R S76N S63Y S67M
GVPMRFYGSGMGTDFTLTINSLRPEDFATYYC

SEQ ID NO: 106 - protein, 32 aa, Artificial Sequence
  FR L3 S81R Q83R S80N S67Y S71M S77R Q79R S76N S63Y S67M
GVPSRFYGSGMGTDFTLTINRLRPEDFATYYC

SEQ ID NO: 107 - protein, 30 aa, Artificial Sequence
  FR L3 S64M S81R Q83R S80N S67Y S71M  S60M S77R Q79R S76N S63Y S67M
PMRFYGSGMGTDFTLTINRLRPEDFATYYC

SEQ ID NO: 108 - protein, 325 aa, Artificial Sequence
  Wild-type human IgE-Fc (CE2-CE4 domains with numbering V224-K547 according to Dorrington & Bennich (1978)
VASRDFTPPTVKILQSSCDGGGHFPPTIQLLCLVSGYTPGTINITWLEDGQVMDVDLSTASTTQEGELASTQSELTLSQKHWLSDRTYTCQVTYQGHTFEDSTKKCADSNPRGVSAYLSRPSPFDLFIRKSPTITCLVVDLAPSKGTVNLTWSRASGKPVNHSTRKEEKQRNGTLTVTSTLPVGTRDWIEGETYQCRVTHPHLPRALMRSTTKTSGPRAAPEVYAFATPEWPGSRDKRTLACLIQNFMPEDISVQWLHNEVQLPDARHSTTQPRKTKGSGFFVFSRLEVTRAEWEQKDEFICRAVHEAASPSQTVQRAVSVNPGK

SEQ ID NO: 109 - protein, 111 aa, Artificial Sequence
  S77R_Q79R_v-region (Fab1)
DIQLTQSPSSLSASVGDRVTITCRASQSVDYDGDSYMNWYQQKPGKAPKLLIYAASYLESGVPSRFSGSGSGTDFTLTISRLRPEDFATYYCQQSHEDPYTFGQGTKVEIK

SEQ ID NO: 110 - DNA, 333 bp, Artificial Sequence
  77R_Q79R_v-region (Fab1)
gatattcagctgactcagagcccgagctcactctccgcttccgtgggggatagagtgaccatcacttgccgggcatcccagtcggtggactacgacggagactcctacatgaactggtaccagcagaagcccggaaaagccccaaagttgctgatctacgccgcctcctaccttgaaagcggcgtgccttcacgcttctcgggaagcgggtctggcaccgatttcaccctgaccatttcgagactgaggccggaggacttcgcgacttactactgccaacagtcccacgaggacccctatacgtttggccagggtaccaaggtcgaaatcaag

SEQ ID NO: 111 - protein, 129 aa, Artificial Sequence
  S77R_Q79R_v-region (Fab1) with signal sequence
MKWVTFISLLFLFSSAYSDIQLTQSPSSLSASVGDRVTITCRASQSVDYDGDSYMNWYQQKPGKAPKLLIYAASYLESGVPSRFSGSGSGTDFTLTISRLRPEDFATYYCQQSHEDPYTFGQGTKVEIK

SEQ ID NO: 112 - DNA, 387 bp, Artificial Sequence
  S77R_Q79R_v-region (Fab1) with signal sequence
atgaagtgggtcaccttcatctccctgctgtttctgttctcctccgcctactccgatattcagctgactcagagcccgagctcactctccgcttccgtgggggatagagtgaccatcacttgccgggcatcccagtcggtggactacgacggagactcctacatgaactggtaccagcagaagcccggaaaagccccaaagttgctgatctacgccgcctcctaccttgaaagcggcgtgccttcacgcttctcgggaagcgggtctggcaccgatttcaccctgaccatttcgagactgaggccggaggacttcgcgacttactactgccaacagtcccacgaggacccctatacgtttggccagggtaccaaggtcgaaatcaag

SEQ ID NO: 113 - protein, 111 aa, Artificial Sequence [sequence omitted]

SEQ ID NO: 114 - DNA, 333 bp, Artificial Sequence; identical to SEQ ID NO: 21
  Fab2_v-region

SEQ ID NO: 115 - protein, 129 aa, Artificial Sequence; identical to SEQ ID NO: 22
  Fab2_v-region with signal sequence

SEQ ID NO: 116 - DNA, 387 bp, Artificial Sequence; identical to SEQ ID NO: 23
  Fab2_v-region with signal sequence

SEQ ID NO: 117 - protein, 218 aa, Artificial Sequence
  Fab2_v-region + kappa constant region including L154P
DIQLTQSPSSLSASVGDRVTITCRASQSVDYDGDSYMNWYQQKPGKAPKLLIYAASYLESGVPSRFSGSGSGTDFTLTISSLQPEDFATYYCQQSHEDPYTFGQGTKVEIKRTVAAPSVFIFPPSDEQLKSGTASVVCLLNNFYPREAKVQWKVDNAPQSGNSQESVTEQDSKDSTYSLSSTLTLSKADYEKHKVYACEVTHQGLSSPVTKSFNRGEC

SEQ ID NO: 118 - DNA, 654 bp, Artificial Sequence
  Fab2_v-region + kappa constant region including L154P
gatattcagctgactcagagcccgagctcactctccgcttccgtgggggatagagtgaccatcacttgccgggcatcccagtcggtggactacgacggagactcctacatgaactggtatcagcagaagcccggaaaagccccaaagttgctgatctacgccgcctcataccttgaaagcggcgtgccttcgcgcttctcgggaagcgggtcgggcaccgatttcaccctgaccatttcgtcgctgcagccggaggacttcgcgacttactactgccaacagtcccacgaggacccctatacgtttggccagggaaccaaggtcgaaatcaagcgtacggtagcggccccatctgtcttcatcttcccgccatctgatgagcagttgaaatctggaactgcctctgttgtgtgcctgctgaataacttctatcccagagaggccaaagtacagtggaaggtggataacgccccgcaatcgggtaactcccaggagagtgtcacagagcaggacagcaaggacagcacctacagcctcagcagcaccctgacgctgagcaaagcagactacgagaaacacaaagtctacgcctgcgaagtcacccatcagggcctgagctcgcccgtcacaaagagcttcaacaggggagagtgt

SEQ ID NO: 119 - protein, 236 aa, Artificial Sequence
  Fab2_v-region + kappa constant region including L154P with signal sequence
MKWVTFISLLFLFSSAYSDIQLTQSPSSLSASVGDRVTITCRASQSVDYDGDSYMNWYQQKPGKAPKLLIYAASYLESGVPSRFSGSGSGTDFTLTISSLQPEDFATYYCQQSHEDPYTFGQGTKVEIKRTVAAPSVFIFPPSDEQLKSGTASVVCLLNNFYPREAKVQWKVDNAPQSGNSQESVTEQDSKDSTYSLSSTLTLSKADYEKHKVYACEVTHQGLSSPVTKSFNRGEC

SEQ ID NO: 120 - DNA, 708 bp, Artificial Sequence
  Fab2_v-region + kappa constant region including L154P with signal sequence
atgaagtgggtcaccttcatctccctgctgtttctgttctcctccgcctactccgatattcagctgactcagagcccgagctcactctccgcttccgtgggggatagagtgaccatcacttgccgggcatcccagtcggtggactacgacggagactcctacatgaactggtatcagcagaagcccggaaaagccccaaagttgctgatctacgccgcctcataccttgaaagcggcgtgccttcgcgcttctcgggaagcgggtcgggcaccgatttcaccctgaccatttcgtcgctgcagccggaggacttcgcgacttactactgccaacagtcccacgaggacccctatacgtttggccagggaaccaaggtcgaaatcaagcgtacggtagcggccccatctgtcttcatcttcccgccatctgatgagcagttgaaatctggaactgcctctgttgtgtgcctgctgaataacttctatcccagagaggccaaagtacagtggaaggtggataacgccccgcaatcgggtaactcccaggagagtgtcacagagcaggacagcaaggacagcacctacagcctcagcagcaccctgacgctgagcaaagcagactacgagaaacacaaagtctacgcctgcgaagtcacccatcagggcctgagctcgcccgtcacaaagagcttcaacaggggagagtgt

SEQ ID NO: 121 - protein, 111 aa, Artificial Sequence; identical to SEQ ID NO: 109
  Fab3_S77R_Q79R_v-region

SEQ ID NO: 122 - DNA, 333 bp, Artificial Sequence; identical to SEQ ID NO: 110
  Fab3_S77R_Q79R_v-region

SEQ ID NO: 123 - protein, 129 aa, Artificial Sequence; identical to SEQ ID NO: 111
  Fab3_S77R_Q79R_v-region with signal sequence

SEQ ID NO: 124 - DNA, 387 bp, Artificial Sequence; identical to SEQ ID NO: 112
  Fab3_S77R_Q79R_v-region with signal sequence

SEQ ID NO: 125 - protein, 218 aa, Artificial Sequence
  Fab3_S77R_Q79R_v-region + kappa constant region including L154P
DIQLTQSPSSLSASVGDRVTITCRASQSVDYDGDSYMNWYQQKPGKAPKLLIYAASYLESGVPSRFSGSGSGTDFTLTISRLRPEDFATYYCQQSHEDPYTFGQGTKVEIKRTVAAPSVFIFPPSDEQLKSGTASVVCLLNNFYPREAKVQWKVDNAPQSGNSQESVTEQDSKDSTYSLSSTLTLSKADYEKHKVYACEVTHQGLSSPVTKSFNRGEC

SEQ ID NO: 126 - DNA, 654 bp, Artificial Sequence
  Fab3_S77R_Q79R_v-region + kappa constant region including L154P
gatattcagctgactcagagcccgagctcactctccgcttccgtgggggatagagtgaccatcacttgccgggcatcccagtcggtggactacgacggagactcctacatgaactggtaccagcagaagcccggaaaagccccaaagttgctgatctacgccgcctcctaccttgaaagcggcgtgccttcacgcttctcgggaagcgggtctggcaccgatttcaccctgaccatttcgagactgaggccggaggacttcgcgacttactactgccaacagtcccacgaggacccctatacgtttggccagggtaccaaggtcgaaatcaagcgtacggtagcggccccatctgtcttcatcttcccgccatctgatgagcagttgaaatctggaactgcctctgttgtgtgcctgctgaataacttctatcccagagaggccaaagtacagtggaaggtggataacgccccgcaatcgggtaactcccaggagagtgtcacagagcaggacagcaaggacagcacctacagcctcagcagcaccctgacgctgagcaaagcagactacgagaaacacaaagtctacgcctgcgaagtcacccatcagggcctgagctcgcccgtcacaaagagcttcaacaggggagagtgt

SEQ ID NO: 127 - protein, 236 aa, Artificial Sequence
  Fab3_S77R_Q79R_v-region + kappa constant region including L154P with signal sequence
MKWVTFISLLFLFSSAYSDIQLTQSPSSLSASVGDRVTITCRASQSVDYDGDSYMNWYQQKPGKAPKLLIYAASYLESGVPSRFSGSGSGTDFTLTISRLRPEDFATYYCQQSHEDPYTFGQGTKVEIKRTVAAPSVFIFPPSDEQLKSGTASVVCLLNNFYPREAKVQWKVDNAPQSGNSQESVTEQDSKDSTYSLSSTLTLSKADYEKHKVYACEVTHQGLSSPVTKSFNRGEC

SEQ ID NO: 128 - DNA, 708 bp, Artificial Sequence
  Fab3_S77R_Q79R_v-region + kappa constant region including L154P with signal sequence
atgaagtgggtcaccttcatctccctgctgtttctgttctcctccgcctactccgatattcagctgactcagagcccgagctcactctccgcttccgtgggggatagagtgaccatcacttgccgggcatcccagtcggtggactacgacggagactcctacatgaactggtaccagcagaagcccggaaaagccccaaagttgctgatctacgccgcctcctaccttgaaagcggcgtgccttcacgcttctcgggaagcgggtctggcaccgatttcaccctgaccatttcgagactgaggccggaggacttcgcgacttactactgccaacagtcccacgaggacccctatacgtttggccagggtaccaaggtcgaaatcaagcgtacggtagcggccccatctgtcttcatcttcccgccatctgatgagcagttgaaatctggaactgcctctgttgtgtgcctgctgaataacttctatcccagagaggccaaagtacagtggaaggtggataacgccccgcaatcgggtaactcccaggagagtgtcacagagcaggacagcaaggacagcacctacagcctcagcagcaccctgacgctgagcaaagcagactacgagaaacacaaagtctacgcctgcgaagtcacccatcagggcctgagctcgcccgtcacaaagagcttcaacaggggagagtgt

SEQ ID NO: 129 - protein, 107 aa, Artificial Sequence
  Omalizumab_v-region
TQSPSSLSASVGDRVTITCRASQSVDYDGDSYMNWYQQKPGKAPKLLIYAASYLESGVPSRFSGSGSGTDFTLTISSLQPEDFATYYCQQSHEDPYTFGQGTKVEIK

SEQ ID NO: 130 - DNA, 321 bp, Artificial Sequence
  Omalizumab_v-region
actcagagcccgagctcactctccgcttccgtgggggatagagtgaccatcacttgccgggcatcccagtcggtggactacgacggagactcctacatgaactggtatcagcagaagcccggaaaagccccaaagttgctgatctacgccgcctcataccttgaaagcggcgtgccttcgcgcttctcgggaagcgggtcgggcaccgatttcaccctgaccatttcgtcgctgcagccggaggacttcgcgacttactactgccaacagtcccacgaggacccctatacgtttggccagggaaccaaggtcgaaatcaag

SEQ ID NO: 131 - protein, 32 aa, Artificial Sequence; identical to SEQ ID NO: 59
  FR3

SEQ ID NO: 132 - protein, 111 aa, Artificial Sequence
  S60M_S52D_S67M_S77R_Q79R_v-region
DIQLTQSPSSLSASVGDRVTITCRASQSVDYDGDSYMNWYQQKPGKAPKLLIYAADYLESGVPMRFSGSGMGTDFTLTISRLRPEDFATYYCQQSHEDPYTFGQGTKVEIK

SEQ ID NO: 133 - DNA, 333 bp, Artificial Sequence
  S60M_S52D_S67M_S77R_Q79R_v-region
gatattcagctgactcagagcccgagctcactctccgcttccgtgggggatagagtgaccatcacttgccgggcatcccagtcggtggactacgacggagactcctacatgaactggtatcagcagaagcccggaaaagccccaaagttgctgatctacgccgccgactaccttgaaagcggcgtgcctatgcgcttctcgggaagcgggatgggcaccgatttcaccctgaccatttcgagactgaggccggaggacttcgcgacttactactgccaacagtcccacgaggacccctatacgtttggccagggaaccaaggtcgaaatcaag

SEQ ID NO: 134 - protein, 129 aa, Artificial Sequence
  S60M_S52D_S67M_S77R_Q79R_v-region with signal sequence
MKWVTFISLLFLFSSAYSDIQLTQSPSSLSASVGDRVTITCRASQSVDYDGDSYMNWYQQKPGKAPKLLIYAADYLESGVPMRFSGSGMGTDFTLTISRLRPEDFATYYCQQSHEDPYTFGQGTKVEIK

SEQ ID NO: 135 - DNA, 387 bp, Artificial Sequence
  S60M_S52D_S67M_S77R_Q79R_v-region with signal sequence
atgaagtgggtcaccttcatctccctgctgtttctgttctcctccgcctactccgatattcagctgactcagagcccgagctcactctccgcttccgtgggggatagagtgaccatcacttgccgggcatcccagtcggtggactacgacggagactcctacatgaactggtatcagcagaagcccggaaaagccccaaagttgctgatctacgccgccgactaccttgaaagcggcgtgcctatgcgcttctcgggaagcgggatgggcaccgatttcaccctgaccatttcgagactgaggccggaggacttcgcgacttactactgccaacagtcccacgaggacccctatacgtttggccagggaaccaaggtcgaaatcaag

SEQ ID NO: 136 - protein, 218 aa, Artificial Sequence
  S60M_S52D_S67M_S77R_Q79R_v-region + kappa constant region
DIQLTQSPSSLSASVGDRVTITCRASQSVDYDGDSYMNWYQQKPGKAPKLLIYAADYLESGVPMRFSGSGMGTDFTLTISRLRPEDFATYYCQQSHEDPYTFGQGTKVEIKRTVAAPSVFIFPPSDEQLKSGTASVVCLLNNFYPREAKVQWKVDNALQSGNSQESVTEQDSKDSTYSLSSTLTLSKADYEKHKVYACEVTHQGLSSPVTKSFNRGEC

SEQ ID NO: 137 - DNA, 654 bp, Artificial Sequence
  S60M_S52D_S67M_S77R_Q79R_v-region + kappa constant region
gatattcagctgactcagagcccgagctcactctccgcttccgtgggggatagagtgaccatcacttgccgggcatcccagtcggtggactacgacggagactcctacatgaactggtatcagcagaagcccggaaaagccccaaagttgctgatctacgccgccgactaccttgaaagcggcgtgcctatgcgcttctcgggaagcgggatgggcaccgatttcaccctgaccatttcgagactgaggccggaggacttcgcgacttactactgccaacagtcccacgaggacccctatacgtttggccagggaaccaaggtcgaaatcaagcgtacggtagcggccccatctgtcttcatcttcccgccatctgatgagcagttgaaatctggaactgcctctgttgtgtgcctgctgaataacttctatcccagagaggccaaagtacagtggaaggtggataacgccctccaatcgggtaactcccaggagagtgtcacagagcaggacagcaaggacagcacctacagcctcagcagcaccctgacgctgagcaaagcagactacgagaaacacaaagtctacgcctgcgaagtcacccatcagggcctgagctcgcccgtcacaaagagcttcaacaggggagagtgt

SEQ ID NO: 138 - protein, 32 aa, Artificial Sequence
  FR3
GVPRRFSGSGMGTDFTLTISRLRPEDFATYYC

SEQ ID NO: 139 - protein, 111 aa, Artificial Sequence
  S60R_S52D_S67M_S77R_Q79R_v-region
DIQLTQSPSSLSASVGDRVTITCRASQSVDYDGDSYMNWYQQKPGKAPKLLIYAADYLESGVPRRFSGSGMGTDFTLTISRLRPEDFATYYCQQSHEDPYTFGQGTKVEIK

SEQ ID NO: 140 - DNA, 333 bp, Artificial Sequence
  S60R_S52D_S67M_S77R_Q79R_v-region
gatattcagctgactcagagcccgagctcactctccgcttccgtgggggatagagtgaccatcacttgccgggcatcccagtcggtggactacgacggagactcctacatgaactggtatcagcagaagcccggaaaagccccaaagttgctgatctacgccgccgattaccttgaaagcggcgtgcctcgtcgcttctcgggaagcgggatgggcaccgatttcaccctgaccatttcgagactgaggccggaggacttcgcgacttactactgccaacagtcccacgaggacccctatacgtttggccagggaaccaaggtcgaaatcaag

SEQ ID NO: 141 - protein, 129 aa, Artificial Sequence
  S60R_S52D_S67M_S77R_Q79R_v-region with signal sequence
MKWVTFISLLFLFSSAYSDIQLTQSPSSLSASVGDRVTITCRASQSVDYDGDSYMNWYQQKPGKAPKLLIYAADYLESGVPRRFSGSGMGTDFTLTISRLRPEDFATYYCQQSHEDPYTFGQGTKVEIK

SEQ ID NO: 142 - DNA, 387 bp, Artificial Sequence
  S60R_S52D_S67M_S77R_Q79R_v-region with signal sequence
atgaagtgggtcaccttcatctccctgctgtttctgttctcctccgcctactccgatattcagctgactcagagcccgagctcactctccgcttccgtgggggatagagtgaccatcacttgccgggcatcccagtcggtggactacgacggagactcctacatgaactggtatcagcagaagcccggaaaagccccaaagttgctgatctacgccgccgattaccttgaaagcggcgtgcctcgtcgcttctcgggaagcgggatgggcaccgatttcaccctgaccatttcgagactgaggccggaggacttcgcgacttactactgccaacagtcccacgaggacccctatacgtttggccagggaaccaaggtcgaaatcaag

SEQ ID NO: 143 - protein, 218 aa, Artificial Sequence
  S60R_S52D_S67M_S77R_Q79R_v-region + kappa constant region
DIQLTQSPSSLSASVGDRVTITCRASQSVDYDGDSYMNWYQQKPGKAPKLLIYAADYLESGVPRRFSGSGMGTDFTLTISRLRPEDFATYYCQQSHEDPYTFGQGTKVEIKRTVAAPSVFIFPPSDEQLKSGTASVVCLLNNFYPREAKVQWKVDNALQSGNSQESVTEQDSKDSTYSLSSTLTLSKADYEKHKVYACEVTHQGLSSPVTKSFNRGEC

SEQ ID NO: 144 - DNA, 654 bp, Artificial Sequence
  S60R_S52D_S67M_S77R_Q79R_v-region + kappa constant region
gatattcagctgactcagagcccgagctcactctccgcttccgtgggggatagagtgaccatcacttgccgggcatcccagtcggtggactacgacggagactcctacatgaactggtatcagcagaagcccggaaaagccccaaagttgctgatctacgccgccgattaccttgaaagcggcgtgcctcgtcgcttctcgggaagcgggatgggcaccgatttcaccctgaccatttcgagactgaggccggaggacttcgcgacttactactgccaacagtcccacgaggacccctatacgtttggccagggaaccaaggtcgaaatcaagcgtacggtagcggccccatctgtcttcatcttcccgccatctgatgagcagttgaaatctggaactgcctctgttgtgtgcctgctgaataacttctatcccagagaggccaaagtacagtggaaggtggataacgccctccaatcgggtaactcccaggagagtgtcacagagcaggacagcaaggacagcacctacagcctcagcagcaccctgacgctgagcaaagcagactacgagaaacacaaagtctacgcctgcgaagtcacccatcagggcctgagctcgcccgtcacaaagagcttcaacaggggagagtgt

SEQ ID NO: 145 - protein, 111 aa, Artificial Sequence
  S60K_S52D_S67M_S77R_Q79R_v-region
DIQLTQSPSSLSASVGDRVTITCRASQSVDYDGDSYMNWYQQKPGKAPKLLIYAADYLESGVPKRFSGSGMGTDFTLTISRLRPEDFATYYCQQSHEDPYTFGQGTKVEIK

SEQ ID NO: 146 - protein, 111 aa, Artificial Sequence
  S60Q_S52D_S67M_S77R_Q79R_v-region
DIQLTQSPSSLSASVGDRVTITCRASQSVDYDGDSYMNWYQQKPGKAPKLLIYAADYLESGVPQRFSGSGMGTDFTLTISRLRPEDFATYYCQQSHEDPYTFGQGTKVEIK

SEQ ID NO: 147 - protein, 506 aa, Artificial Sequence
  v-region + gamma 1 CH1 constant region plus linker plus CA645 gL4gH5 scFv with signal sequence
MKWVTFISLLFLFSSAYSEVQLVESGGGLVQPGGSLRLSCAVSGYSITSGYSWNWIRQAPGKGLEWVASITYDGSTNYNPSVKGRITISRDDSKNTFYLQMNSLRAEDTAVYYCARGSHYFGHWHFAVWGQGTLVTVSSASTKGPSVFPLAPSSKSTSGGTAALGCLVKDYFPEPVTVSWNSGALTSGVHTFPAVLQSSGLYSLSSVVTVPSSSLGTQTYICNVNHKPSNTKVDKKVEPKSCSGGGGTGGGGSEVQLLESGGGLVQPGGSLRLSCAVSGIDLSNYAINWVRQAPGKCLEWIGIIWASGTTFYATWAKGRFTISRDNSKNTVYLQMNSLRAEDTAVYYCARTVPGYSTAPYFDLWGQGTLVTVSSGGGGSGGGGSGGGGSGGGGSDIQMTQSPSSVSASVGDRVTITCQSSPSVWSNFLSWYQQKPGKAPKLLIYEASKLTSGVPSRFSGSGSGTDFTLTISSLQPEDFATYYCGGGYSSISDTTFGCGTKVEIKRT

SEQ ID NO: 148 - DNA, 1518 bp, Artificial Sequence
  v-region + gamma 1 CH1 constant region plus linker plus CA645 gL4gH5 scFv with signal sequence
atgaagtgggtcaccttcatctccctgctgtttctgttctccagcgcctactccgaagtgcagttggtggagtcgggtggagggctggtgcagcctggcggtagcctgaggctgtcctgtgccgtgtccggatactccattacctccggctactcgtggaactggatcagacaggctcccggaaagggacttgagtgggtggcgtccatcacctacgacggctcaaccaactataacccgtccgtgaagggccgcatcaccatttcgcgcgacgacagcaagaatactttttacctccaaatgaacagcctgcgggccgaagatactgccgtgtactactgcgcgcggggatcacattacttcgggcactggcacttcgccgtctggggacagggcaccctcgtcactgtctcgagcgcttctacaaagggcccatcggtcttccccctggcaccctcctccaagagcacctctgggggcacagcggccctgggctgcctggtcaaggactacttccccgaaccagtgacggtgtcgtggaactcaggtgccctgaccagcggcgttcacaccttcccggctgtcctacagtcttcaggactctactccctgagcagcgtggtgaccgtgccctccagcagcttgggcacccagacctacatctgcaacgtgaatcacaagcccagcaacaccaaggtcgataagaaagttgagcccaaatcttgtagtggaggtgggggcaccggtggaggtggcagcgaggttcaactgcttgagtctggaggaggcctagtccagcctggagggagcctgcgtctctcttgtgcagtaagcggcatcgacctgagcaattacgccatcaactgggtgagacaagctccggggaagtgtttagaatggatcggtataatatgggccagtgggacgaccttttatgctacatgggcgaaaggaaggtttacaattagccgggacaatagcaaaaacaccgtgtatctccaaatgaactccttgcgagcagaggacacggcggtgtactattgtgctcgcactgtcccaggttatagcactgcaccctacttcgatctgtggggacaagggaccctggtgactgtttcaagtggcggagggggtagtggagggggtggctctgggggtggcggaagcggtggcgggggttctgacatacaaatgactcagtctccttcatcggtatccgcgtccgttggcgatagggtgactattacatgtcaaagctctcctagcgtctggagcaattttctatcctggtatcaacagaaaccggggaaggctccaaaacttctgatttatgaagcctcgaaactcaccagtggagttccgtcaagattcagtggctctggatcagggacagacttcacgttgacaatcagttcgctgcaaccagaggactttgcgacctactattgtggtggaggttacagtagcataagtgatacgacatttgggtgcggtactaaggtggaaatcaaacgtacc

SEQ ID NO: 149 - protein, 11 aa, Artificial Sequence
  Linker between CH1 and CA645 gL4gH5 scFv
SGGGGTGGGGS

SEQ ID NO: 150 - protein, 253 aa, Artificial Sequence
  CA645 gL4gH5 scFv
EVQLLESGGGLVQPGGSLRLSCAVSGIDLSNYAINWVRQAPGKCLEWIGIIWASGTTFYATWAKGRFTISRDNSKNTVYLQMNSLRAEDTAVYYCARTVPGYSTAPYFDLWGQGTLVTVSSGGGGSGGGGSGGGGSGGGGSDIQMTQSPSSVSASVGDRVTITCQSSPSVWSNFLSWYQQKPGKAPKLLIYEASKLTSGVPSRFSGSGSGTDFTLTISSLQPEDFATYYCGGGYSSISDTTFGCGTKVEIKRT

SEQ ID NO: 151 - protein, 20 aa, Artificial Sequence
  Linker between CA645 gH5 and CA645 gL4 within scFv
GGGGSGGGGSGGGGSGGGGS

SEQ ID NO: 152 - protein, 10 aa, Artificial Sequence
  CA645 CDRH1
GIDLSNYAIN

SEQ ID NO: 153 - protein, 16 aa, Artificial Sequence
  CA645 CDRH2
IIWASGTTFYATWAKG

SEQ ID NO: 154 - protein, 13 aa, Artificial Sequence
  CA645 CDRH3
TVPGYSTAPYFDL

SEQ ID NO: 155 - protein, 12 aa, Artificial Sequence
  CA645 CDRL1
QSSPSVWSNFLS

SEQ ID NO: 156 - protein, 7 aa, Artificial Sequence
  CA645 CDRL2
EASKLTS

SEQ ID NO: 157 - protein, 10 aa, Artificial Sequence
  CA645 CDRL3
GGYSSISDTT

SEQ ID NO: 158 - protein, 111 aa, Artificial Sequence
  S60M_S52D_S67M_S77R_Q79R_S63W_S76N_v-region
DIQLTQSPSSLSASVGDRVTITCRASQSVDYDGDSYMNWYQQKPGKAPKLLIYAADYLESGVPMRFWGSGMGTDFTLTINRLRPEDFATYYCQQSHEDPYTFGQGTKVEIK

SEQ ID NO: 159 - protein, 111 aa, Artificial Sequence
  S60M_S52D_S67M_S77R_Q79R_S63Y_S76N_v-region
DIQLTQSPSSLSASVGDRVTITCRASQSVDYDGDSYMNWYQQKPGKAPKLLIYAADYLESGVPMRFYGSGMGTDFTLTINRLRPEDFATYYCQQSHEDPYTFGQGTKVEIK

SEQ ID NO: 160 - protein, 18 aa, Artificial Sequence
  Signal sequence
MKWVTFISLLFLFSSAYS